European Patent Specification EP 4 135 755 B1, published June 25, 2025. Title: Compositions and methods for treating hair follicle-linked conditions. Applicant: Henlez ApS. The sequence listing filed with the application follows.

SEQUENCE LISTING (14 sequences)

SEQ ID NO: 1 - protein, 222 aa, Bacillus licheniformis
SVIGSDDRTRVTNTTAYPYRAIVHISSSIGSCTGWMIGPKTVATAGHCIYDTSSGSFAGTATVSPGRNGTSYPYGSVKSTRYFIPSGWRSGNTNYDYGAIELSEPIGNTVGYFGYSYTTSSLVGTTVTISGYPGDKTAGTQWQHSGPIAISETYKLQYAMDTYGGQSGSPVFEQSSSRTNCSGPCSLAVHTNGVYGGSSYNRGTRITKEVFDNLTNWKNSAQ

SEQ ID NO: 2 - protein, 274 aa, Bacillus licheniformis
AQTVPYGIPLIKADKVQAQGFKGANVKVAVLDTGIQASHPDLNVVGGASFVAGEAYNTDGNGHGTHVAGTVAALDNTTGVLGVAPSVSLYAVKVLNSSGSGSYSGIVSGIEWATTNGMDVINMSLGGASGSTAMKQAVDNAYARGVVVVAAAGNSGSSGNTNTIGYPAKYDSVIAVGAVDSNSNRASFSSVGAELEVMAPGAGVYSTYPTNTYATLNGTSMASPHVAGAAALILSKHPNLSASQVRNRLSSTATYLGSSFYYGKGLINVEAAAQ

SEQ ID NO: 3 - protein, 268 aa, Achromobacter lyticus
GVSGSCNIDVVCPEGDGRRDIIRAVGAYSKSGTLACTGSLVNNTANDRKMYFLTAHHCGMGTASTAASIVVYWNYQNSTCRAPNTPASGANGDGSMSQTQSGSTVKATYATSDFTLLELNNAANPAFNLFWAGWDRRDQNYPGAIAIHHPNVAEKRISNSTSPTSFVAWGGGAGTTHLNVQWQPSGGVTEPGSSGSPIYSPEKRVLGQLHGGPSSCSATGTNRSDQYGRVFTSWTGGGAAASRLSDWLDPASTGAQFIDGLDSGGGTP

SEQ ID NO: 4 - protein, 268 aa, Bacillus halodurans
QTVPWGISFINTQQAHNRGIFGNGARVAVLDTGIASHPDLRIAGGASFISSEPSYHDNNGHGTHVAGTIAALNNSIGVLGVAPSADLYAVKVLDRNGSGSLASVAQGIEWAINNNMHIINMSLGSTSGSSTLELAVNRANNAGILLVGAAGNTGRQGVNYPARYSGVMAVAAVDQNGQRASFSTYGPEIEISAPGVNVNSTYTGNRYVSLSGTSMATPHVAGVAALVKSRYPSYTNNQIRQRINQTATYLGSPSLYGNGLVHAGRATQ

SEQ ID NO: 5 - protein, 342 aa, Saccharothrix variesporea
AGETAGALATACATGTWGYLDHDGVARVSPNAKVWAYDDDANGADDLLATGLTDGNGRFNLCYDNTDDEGGGQDVYVRTATENTLWIIRNGRTRKSYSFYTDVIANGGSAVDFGTVRPSDPALMRGVEAFDTVNAAWNWTPGNCWDARDTTCRQGKINWAPDSTDGTYYSLQENAVHLAAEDPDSNILVLHEFGHYMMDDVYEDDFPPAPNCSPHYITKISSAGCAWTEGFATWFGVAVLGDPTFRWPGGRTLDLEGPTWGTANWDNGDTVEGRVLGSMIDLYDTTNEPGDTCSENPAGPLWTTFLNHVSDTFAQYWSHRRADGYDVGSNALSCLYHNTIDY

SEQ ID NO: 6 - protein, 300 aa, Bacillus amyloliquefaciens
AATTGTGTTLKGKTVSLNISSESGKYVLRDLSKPTGTQIITYDLQNREYNLPGTLVSSTTNQFTTSSQRAAVDAHYNLGKVYDYFYQKFNRNSYDNKGGKIVSSVHYGSRYNNAAWIGDQMIYGDGDGSFFSPLSGSMDVTAHEMTHGVTQETANLNYENQPGALNESFSDVFGYFNDTEDWDIGEDITVSQPALRSLSNPTKYGQPDNFKNYKNLPNTDAGDYGGVHTNSGIPNKAAYNTITKIGVNKAEQIYYRALTVYLTPSSTFKDAKAALIQSARDLYGSQDAASVEAAWNAVGL

SEQ ID NO: 7 - protein, 269 aa, Bacillus clausii
AQSVPWGIERVQAPAAHNRGLTGSGVKVAVLDTGISTHPDLRIRGGASFVPGEPSTQDGNGHGTHVAGTIAALDNSIGVLGVAPSEALYAVKVLGASGSGSVSSIAQGLEWAGNNGMHVANLSLGSPSPSATLEQAVNSATSRGVLVVAASGNSGAGSISYPARYANAMAVGATDQNNNRASFSQYGAGLDIVAPGVNILSTWPGSTYASLNGTSMATPHVAGAAALVKQKNPSWSNVQIRNHLKNTATSLGDTWEYGSGLVNAEAATR

SEQ ID NO: 8 - protein, 188 aa, Nocardiopsis sp NRRL 18262
ADIIGGLAYTMGGRCSVGFAATNAAGQPGFVTAGHCGRVGTQVTIGNGRGVFEQSVFPGNDAAFVRGTSNFTLTNLVSRYNTGGYATVAGHNQAPIGSSVCRSGSTTGWHCGTIQARGQSVSYPEGTVTNMTRTTVCAEPGDSGGSYISGTQAQGVTSGGSGNCRTGGTTFYQEVTPMVNSWGVRLRT

SEQ ID NO: 9 - protein, 185 aa, Streptomyces coelicolor
YQPSAGSGEDAAANRAFFEAVVKSVAEKRAANPSAAAAVTVYYSATNAPSFRSQISRSAQIWNSSVSNVRLAESSSGADFAYYEGNDSRGSYASTDGHGSGYIFLDYRQNQQYDSTRVTAHETGHVLGLPDHYSGPCSELMSGGGPGPSCTNPYPNSTERSRVNQLWAYGFQAALDKALEKASQR

SEQ ID NO: 10 - protein, 224 aa, Fusarium oxysporum
IVGGTSASAGDFPFIVSISRNGGPWCGGSLLNANTVLTAAHCVSGYAQSGFQIRAGSLSRTSGGITSSLSSVRVHPSYSGNNNDLAILKLSTSIPSGGNIGYARLAASGSDPVAGSSATVAGWGATSEGGSSTPVNLLKVTVPIVSRATCRAQYGTSAITNQMFCAGVSSGGKDSCQGDSGGPIVDSSNTLIGAVSWGNGCARPNYSGVYASVGALRSFIDTYA

SEQ ID NO: 11 - protein, 178 aa, Thermoascus aurantiacus
RTRISSCSGSRQSALTTALRNAASLANAAADAAQSGSASKFSEYFKTTSSSTRQTVAARLRAVAREASSSSSGATTYYCDDPYGYCSSNVLAYTLPSYNIIANCDIFYTYLPALTSTCHAQDQATTALHEFTHAPGVYSPGTDDLAYGYQAAMGLSSSQAVMNADTYALYANAIYLGC

SEQ ID NO: 12 - protein, 187 aa, Streptomyces griseus
VLGGGAIYGGGSRCSAAFNVTKGGARYFVTAGHCTNISANWSASSGGSVVGVREGTSFPTNDYGIVRYTDGSSPAGTVDLYNGSTQDISSAANAVVGQAIKKSGSTTKVTSGTVTAVNVTVNYGDGPVYNMVRTTACSAGGDSGGAHFAGSVALGIHSGSSGCSGTAGSAIHQPVTEALSAYGVTVY

SEQ ID NO: 13 - protein, 215 aa, Bacillus pumilus JA16
VVIGDDGRTKVTNTRVAPYNSIAYITFGGSSCTGTLIAPNKILTNGHCVYNTATRSYSAKGSVYPGMNDSTAVNGSANMTEFYVPSGYINTGASQYDFAVIKTDTNIGNTVGYRSIRQVTNLTGTTIKISGYPGDKMRSTGKVSQWEMSGPVTREDTNLAYYTIDTFSGNSGSAMLDQNQQIVGVHNAGYSNGTINGGPKATAAFVEFINYAKAQ

SEQ ID NO: 14 - protein, 268 aa, Staphylococcus aureus
VILPNNDRHQITDTTNGHYAPVTYIQVEAPTGTFIASGVVVGKDTLLTNKHVVDATHGDPHALKAFPSAINQDNYPNGGFTAEQITKYSGEGDLAIVKFSPNEQNKHIGEVVKPATMSNNAETQVNQNITVTGYPGDKPVATMWESKGKITYLKGEAMQYDLSTTGGNSGSPVFNEKNEVIGIHWGGVPNEFNGAVFINENVRNFLKQNIEDIHFANDDQPNNPDNPDNPNNPDNPNNPDEPNNPDNPNNPDNPDNGDNNNSDNPDAA